European Patent Specification EP 3 696 195 B1, published February 14, 2024. Title: ANTI-DESPR INHIBITORS AS THERAPEUTICS FOR INHIBITION OF PATHOLOGICAL ANGIOGENESIS AND TUMOR CELL INVASIVENESS AND FOR MOLECULAR IMAGING AND TARGETED DELIVERY. Applicant: TRUSTEES OF BOSTON UNIVERSITY. Application PCT/US11/45056. The sequence listing filed with the application follows.

SEQUENCE LISTING (27 sequences)

SEQ ID NO: 1 - protein, 85 aa, Homo sapiens
MTMFKGSNEMKSRWNWGSITCIICFTCVGSQLSMSSSKASNFSGPLQLYQRELEIFIVLTDVPNYRLIKENSHLHTTIVDQGRTV

SEQ ID NO: 2 - protein, 26 aa, Homo sapiens
MNFLLSWVHWSLALLLYLHHAKWSQA

SEQ ID NO: 3 - DNA, 357 bp, Artificial Sequence
  source: /note="Description of Artificial Sequence: Synthetic polynucleotide"
  CDS (1)..(357)
caggtgcaactgaaggagtcaggacctggcctggtggcgccctcacagagcctgtccattacctgcactgtctctgggttctcattaaccagctatgatataagctggattcgccagccaccaggaaagggtctggagtggcttggagtaatatggactggtggaggcacaaattataattcagctttcatgtccagactgagcatcagcaaggacaactccaagagccaagttttcttaaaaatgaacagtctgcaaactgatgacacagccatatattactgtgtaagagatcgggattacgacgggtggtacttcgatgtctggggcgcagggaccacggtcaccgtctcctca

SEQ ID NO: 4 - protein, 119 aa, Artificial Sequence
  source: /note="Description of Artificial Sequence: Synthetic polypeptide"
QVQLKESGPGLVAPSQSLSITCTVSGFSLTSYDISWIRQPPGKGLEWLGVIWTGGGTNYNSAFMSRLSISKDNSKSQVFLKMNSLQTDDTAIYYCVRDRDYDGWYFDVWGAGTTVTVSS

SEQ ID NO: 5 - protein, 10 aa, Artificial Sequence
  source: /note="Description of Artificial Sequence: Synthetic peptide"
GFSLTSYDIS

SEQ ID NO: 6 - protein, 16 aa, Artificial Sequence
  source: /note="Description of Artificial Sequence: Synthetic peptide"
VIWTGGGTNYNSAFMS

SEQ ID NO: 7 - protein, 11 aa, Artificial Sequence
  source: /note="Description of Artificial Sequence: Synthetic peptide"
DRDYDGWYFDV

SEQ ID NO: 8 - DNA, 336 bp, Artificial Sequence
  source: /note="Description of Artificial Sequence: Synthetic polynucleotide"
  CDS (1)..(336)
gatgttttgatgacccaaactccactctccctgcctgtcagtcttggagatcaagcctccatctcttgcagatctagtcagagcattgtacatagtaatggaaacacctatttagaatggtacctgcagaaaccaggccagtctccaaagctcctgatctacaaagtttccaaccgattttctggggtcccagacaggttcagtggcagtggatcagggacagatttcacactcaagatcagcagagtggaggctgaggatctgggagtttattactgctttcaaggttcacatgttccgtacacgttcggaggggggaccaagctggaaataaaa

SEQ ID NO: 9 - protein, 112 aa, Artificial Sequence
  source: /note="Description of Artificial Sequence: Synthetic polypeptide"
DVLMTQTPLSLPVSLGDQASISCRSSQSIVHSNGNTYLEWYLQKPGQSPKLLIYKVSNRFSGVPDRFSGSGSGTDFTLKISRVEAEDLGVYYCFQGSHVPYTFGGGTKLEIK

SEQ ID NO: 10 - protein, 16 aa, Artificial Sequence
  source: /note="Description of Artificial Sequence: Synthetic peptide"
RSSQSIVHSNGNTYLE

SEQ ID NO: 11 - protein, 7 aa, Artificial Sequence
  source: /note="Description of Artificial Sequence: Synthetic peptide"
KVSNRFS

SEQ ID NO: 12 - protein, 9 aa, Artificial Sequence
  source: /note="Description of Artificial Sequence: Synthetic peptide"
FQGSHVPYT

SEQ ID NO: 13 - protein, 119 aa, Artificial Sequence
  source: /note="Description of Artificial Sequence: Synthetic polypeptide"
QVQLQESGPGLVKPSQTLSLTCTVSGFSLTSYDISWIRQPPGKGLEWLGVIWTGGGTNYNSAFMSRLTISKDNSKSTVYLQMNSLRAEDTAIYYCVRDRDYDGWYFDVWGQGTTVTVSS

SEQ ID NO: 14 - protein, 119 aa, Artificial Sequence
  source: /note="Description of Artificial Sequence: Synthetic polypeptide"
QVQLQESGPGLVKPSQTLSLTCTVSGFSLTSYDISWIRQPPGKGLEWLGVIWTGGGTNYNSAFMSRLTISKDNSKNTVYLQMNSLRAEDTAIYYCVRDRDYDGWYFDVWGQGTTVTVSS

SEQ ID NO: 15 - protein, 119 aa, Artificial Sequence
  source: /note="Description of Artificial Sequence: Synthetic polypeptide"
QVQLQESGPGLVKPSQTLSLTCTVSGFSLTSYDISWIRQPPGKGLEWLGVIWTGGGTNYNSAFMSRFTISKDNSKNTVYLQMNSLRAEDTAIYYCVRDRDYDGWYFDVWGQGTTVTVSS

SEQ ID NO: 16 - protein, 119 aa, Artificial Sequence
  source: /note="Description of Artificial Sequence: Synthetic polypeptide"
QVQLQESGPGLVKPSQTLSLTCTVSGFSLTSYDISWIRQPPGKGLEWLGVIWTGGGTNYNSAFMSRLTISKDNSKNTVYLQMNSLRAEDTAVYYCVRDRDYDGWYFDVWGQGTTVTVSS

SEQ ID NO: 17 - protein, 119 aa, Artificial Sequence
  source: /note="Description of Artificial Sequence: Synthetic polypeptide"
QVQLQESGPGLVKPSQTLSLTCTVSGFSLTSYDISWIRQPPGKGLEWLGVIWTGGGTNYNSAFMSRFTISKDNSKNTVYLQMNSLRAEDTAVYYCVRDRDYDGWYFDVWGQGTTVTVSS

SEQ ID NO: 18 - protein, 112 aa, Artificial Sequence
  source: /note="Description of Artificial Sequence: Synthetic polypeptide"
DVLMTQSPLSLPVTLGQPASISCRSSQSIVHSNGNTYLEWYLQKPGQSPQLLIYKVSNRFSGVPDRFSGSGSGTDFTLKISRVEAEDVGVYYCFQGSHVPYTFGQGTKLEIK

SEQ ID NO: 19 - protein, 112 aa, Artificial Sequence
  source: /note="Description of Artificial Sequence: Synthetic polypeptide"
DVVMTQSPLSLPVTLGQPASISCRSSQSIVHSNGNTYLEWYLQKPGQSPQLLIYKVSNRFSGVPDRFSGSGSGTDFTLKISRVEAEDVGVYYCFQGSHVPYTFGQGTKLEIK

SEQ ID NO: 20 - protein, 9 aa, Homo sapiens
MTMFKGSNE

SEQ ID NO: 21 - DNA, 357 bp, Artificial Sequence
  source: /note="Description of Artificial Sequence: Synthetic polynucleotide"
  CDS (1)..(357)
caggtgcagctgcaggagagcggccctggcctggtgaagcctagccagaccctgagcctgacctgcaccgtgagcggcttcagcctgaccagctacgacatcagctggatcagacagcctcctggcaagggcctggagtggctgggcgtgatctggaccggcggcggcaccaactacaacagcgccttcatgagcagactgaccatcagcaaggacaacagcaagagcaccgtgtacctgcagatgaacagcctgagagccgaggacaccgccatctactactgcgtgagagacagagactacgacggctggtacttcgacgtgtggggccagggcaccaccgtgaccgtgagcagc

SEQ ID NO: 22 - DNA, 357 bp, Artificial Sequence
  source: /note="Description of Artificial Sequence: Synthetic polynucleotide"
  CDS (1)..(357)
caggtgcagctgcaggagagcggccctggcctggtgaagcctagccagaccctgagcctgacctgcaccgtgagcggcttcagcctgaccagctacgacatcagctggatcagacagcctcctggcaagggcctggagtggctgggcgtgatctggaccggcggcggcaccaactacaacagcgccttcatgagcagactgaccatcagcaaggacaacagcaagaacaccgtgtacctgcagatgaacagcctgagagccgaggacaccgccatctactactgcgtgagagacagagactacgacggctggtacttcgacgtgtggggccagggcaccaccgtgaccgtgagcagc

SEQ ID NO: 23 - DNA, 357 bp, Artificial Sequence
  source: /note="Description of Artificial Sequence: Synthetic polynucleotide"
  CDS (1)..(357)
caggtgcagctgcaggagagcggccctggcctggtgaagcctagccagaccctgagcctgacctgcaccgtgagcggcttcagcctgaccagctacgacatcagctggatcagacagcctcctggcaagggcctggagtggctgggcgtgatctggaccggcggcggcaccaactacaacagcgccttcatgagcagattcaccatcagcaaggacaacagcaagaacaccgtgtacctgcagatgaacagcctgagagccgaggacaccgccatctactactgcgtgagagacagagactacgacggctggtacttcgacgtgtggggccagggcaccaccgtgaccgtgagcagc

SEQ ID NO: 24 - DNA, 357 bp, Artificial Sequence
  source: /note="Description of Artificial Sequence: Synthetic polynucleotide"
  CDS (1)..(357)
caggtgcagctgcaggagagcggccctggcctggtgaagcctagccagaccctgagcctgacctgcaccgtgagcggcttcagcctgaccagctacgacatcagctggatcagacagcctcctggcaagggcctggagtggctgggcgtgatctggaccggcggcggcaccaactacaacagcgccttcatgagcagactgaccatcagcaaggacaacagcaagaacaccgtgtacctgcagatgaacagcctgagagccgaggacaccgccgtgtactactgcgtgagagacagagactacgacggctggtacttcgacgtgtggggccagggcaccaccgtgaccgtgagcagc

SEQ ID NO: 25 - DNA, 357 bp, Artificial Sequence
  source: /note="Description of Artificial Sequence: Synthetic polynucleotide"
  CDS (1)..(357)
caggtgcagctgcaggagagcggccctggcctggtgaagcctagccagaccctgagcctgacctgcaccgtgagcggcttcagcctgaccagctacgacatcagctggatcagacagcctcctggcaagggcctggagtggctgggcgtgatctggaccggcggcggcaccaactacaacagcgccttcatgagcagattcaccatcagcaaggacaacagcaagaacaccgtgtacctgcagatgaacagcctgagagccgaggacaccgccgtgtactactgcgtgagagacagagactacgacggctggtacttcgacgtgtggggccagggcaccaccgtgaccgtgagcagc

SEQ ID NO: 26 - DNA, 336 bp, Artificial Sequence
  source: /note="Description of Artificial Sequence: Synthetic polynucleotide"
  CDS (1)..(336)
gacgtgctgatgacccagagccctctgagcctgcctgtgaccctgggccagcctgccagcatcagctgcagaagcagccagagcatcgtgcacagcaacggcaacacctacctggagtggtacctgcagaagcctggccagagccctcagctgctgatctacaaggtgagcaacagattcagcggcgtgcctgacagattcagcggcagcggcagcggcaccgacttcaccctgaagatcagcagagtggaggccgaggacgtgggcgtgtactactgcttccagggcagccacgtgccttacaccttcggccagggcaccaagctggagatcaag

SEQ ID NO: 27 - DNA, 336 bp, Artificial Sequence
  source: /note="Description of Artificial Sequence: Synthetic polynucleotide"
  CDS (1)..(336)
gacgtggtgatgacccagagccctctgagcctgcctgtgaccctgggccagcctgccagcatcagctgcagaagcagccagagcatcgtgcacagcaacggcaacacctacctggagtggtacctgcagaagcctggccagagccctcagctgctgatctacaaggtgagcaacagattcagcggcgtgcctgacagattcagcggcagcggcagcggcaccgacttcaccctgaagatcagcagagtggaggccgaggacgtgggcgtgtactactgcttccagggcagccacgtgccttacaccttcggccagggcaccaagctggagatcaag